European Patent Application EP 4 234 576 A2, published August 30, 2023. Title: METHODS OF ISOLATING NEOANTIGEN-SPECIFIC T CELL RECEPTOR SEQUENCES. Applicant: THE UNITED STATES OF AMERICA, AS REPRESENTED BY THE SECRETARY, DEPARTMENT OF HEALTH AND HUMAN SERVICES. The sequence listing filed with the application follows.

SEQUENCE LISTING (25 sequences)

SEQ ID NO: 1 - protein, 27 aa, Homo sapiens
RAKRSGSGATNFSLLKQAGDVEENPGP

SEQ ID NO: 2 - protein, 25 aa, Homo sapiens
WAKFLDPITGTFHYYHSPTNTVHMY

SEQ ID NO: 3 - protein, 9 aa, Homo sapiens
GADGVGKSA

SEQ ID NO: 4 - protein, 10 aa, Homo sapiens
WSYDSTLLAY

SEQ ID NO: 5 - skipped

SEQ ID NO: 6 - DNA, 39 bp, Homo sapiens
  source 1..39: mol_type = other DNA
tgtgctgtgagagaccatagcaactatcagttaatctgg

SEQ ID NO: 7 - protein, 13 aa, Homo sapiens
CAVRDHSNYQLIW

SEQ ID NO: 8 - DNA, 54 bp, Homo sapiens
  source 1..54: mol_type = other DNA
tgtgccagcagccaatccggtgggggcgggttctcctacaatgagcagttcttc

SEQ ID NO: 9 - protein, 18 aa, Homo sapiens
CASSQSGGGGFSYNEQFF

SEQ ID NO: 10 - DNA, 45 bp, Homo sapiens
  source 1..45: mol_type = other DNA
tgcctcgtgggtgacatggaccaggcaggaactgctctgatcttt

SEQ ID NO: 11 - protein, 15 aa, Homo sapiens
CLVGDMDQAGTALIF

SEQ ID NO: 12 - DNA, 45 bp, Homo sapiens
  source 1..45: mol_type = other DNA
tgtgccagcagcttggggagggcaagcaatcagccccagcatttt

SEQ ID NO: 13 - protein, 15 aa, Homo sapiens
CASSLGRASNQPQHF

SEQ ID NO: 14 - DNA, 39 bp, Homo sapiens
  source 1..39: mol_type = other DNA
tgtgctttcatgtggggattaggtcagaattttgtcttt

SEQ ID NO: 15 - protein, 13 aa, Homo sapiens
CAFMWGLGQNFVF

SEQ ID NO: 16 - DNA, 45 bp, Homo sapiens
  source 1..45: mol_type = other DNA
tgtgccagcagtgtggagcgggagaacaccggggagctgtttttt

SEQ ID NO: 17 - protein, 15 aa, Homo sapiens
CASSVERENTGELFF

SEQ ID NO: 18 - protein, 14 aa, Homo sapiens
VWDALFADGLSLCL

SEQ ID NO: 19 - protein, 13 aa, Homo sapiens
WRRVAWSYDSTLL

SEQ ID NO: 20 - protein, 8 aa, Homo sapiens
WSYDSTLL

SEQ ID NO: 21 - protein, 9 aa, Homo sapiens
WSYDSTLLA

SEQ ID NO: 22 - protein, 10 aa, Homo sapiens
WSYDSTLLAY

SEQ ID NO: 23 - protein, 12 aa, Homo sapiens
YLALVDKNIIGY

SEQ ID NO: 24 - protein, 9 aa, Homo sapiens
YSEPDVSGK

SEQ ID NO: 25 - protein, 25 aa, Homo sapiens
LGKFPELFNWFKIFLGYKESVHLET